European Patent Application EP 4 218 796 A1, published August 2, 2023. Title: Antibacterial properties of polypeptides with NlpC/P60 domains. Applicant: Philipps-Universität Marburg. The sequence listing filed with the application follows.

SEQUENCE LISTING (42 sequences)

SEQ ID NO: 1 - protein, 119 aa, Unknown
  NlpC/P60 domain of LytF
SAKINTMISAAKAQLGVPYRWGGTTPSGFDCSGFIYYVLNKVTSVSRLTAAGYWNTMKSVSQPAVGDFVFFSTYKAGPSHVGIYLGNGEFINANDSGVVISNMNNSYWKQRYLGAKRYF

SEQ ID NO: 2 - protein, 93 aa, Unknown
  CHAP domain of LysK endolysin
IDADGYYHAQCQDLITDYVLWLTDNKVRTWGNAKDQIKQSYGTGFKIHENKPSTVPKKGWIAVFTSGSYEQWGHIGIVYDGGNTSTFTILEQN

SEQ ID NO: 3 - DNA, 1386 bp, Artificial Sequence
  LytF without signal peptide
gcaacgattaaggtcaaaagcggagattctttatggaaactggcccaaacctataacacaagtgtggcggccctcacatccgccaatcatctttcgactactgttctgtcgatcggccagacgcttactattccaggcagcaaatccagcacttcttcatctacttcaagctcaacaaccaagaagagcggaagttctgtttacacagtgaaaagcggagattcactttggctgatcgcaaatgagtttaaaatgacggtgcaggaactgaaaaaattaaacggactaagcagcgatttaattcgtgctgggcagaaattaaaggtgtccggtactgtttcttcaagctctagttccagtaaaaaaagcaactctaataagagttcaagctccagttcaaaaagcagttctaataagagttcaagttcttcatcttctacgggaacatataaggtgcagcttggagattcactttggaaaattgcaaacaaagtcaatatgtccatcgctgaattgaaggtcttgaacaacttaaaatcagacaccatttacgtgaatcaggtgttgaaaacaaaatcaagcggctctgatacgtcttctaaagacaattcatccaaatcgaaccaaacttcagcaacaactaaatataccgttaaaagcggtgattcactttggaaaatcgcaaacaactataacctgactgtacagcaaatccgaaatatcaacaatctgaaatcagatgtgctttacgttggacaagtattgaagctgacaggtaaagcatcttcaggctcttcatcatcgtcgtcttcttcgtcaaatgcaagctccggcacgacgactacatacacggtgaaaagcggtgattccttatgggtgattgctcaaaaatttaatgtaacagctcagcagattcgtgagaaaaacaatttaaaaacggatgtcttgcaggttggccaaaagctggtcatttccggaaaagcttcatcatcgtcttcatccggttcttcaaacaccaccagctcaacgagtgcgaagattaacacaatgatttcggccgctaaagcgcagcttggggttccgtatcgctggggaggcacgacaccgtccgggtttgactgcagcggattcatttactatgtactgaacaaagtcacatccgtatctagattaacggcagcgggatattggaacacaatgaaatcagttagccagcctgctgtcggagatttcgttttcttttcaacatataaagccggcccttcccacgtcggaatttacctaggcaacggggaattcataaatgccaacgattccggagttgtcatttccaatatgaacaactcttactggaaacagcgctatctcggtgcaaaacgatatttc

SEQ ID NO: 4 - protein, 26 aa, Unknown
  LytF signal peptide
MKKKLAAGLTASAIVGTTLVVTPAEA

SEQ ID NO: 5 - protein, 488 aa, Unknown
  LytF protein
MKKKLAAGLTASAIVGTTLVVTPAEAATIKVKSGDSLWKLAQTYNTSVAALTSANHLSTTVLSIGQTLTIPGSKSSTSSSTSSSTTKKSGSSVYTVKSGDSLWLIANEFKMTVQELKKLNGLSSDLIRAGQKLKVSGTVSSSSSSSKKSNSNKSSSSSSKSSSNKSSSSSSSTGTYKVQLGDSLWKIANKVNMSIAELKVLNNLKSDTIYVNQVLKTKSSGSDTSSKDNSSKSNQTSATTKYTVKSGDSLWKIANNYNLTVQQIRNINNLKSDVLYVGQVLKLTGKASSGSSSSSSSSSNASSGTTTTYTVKSGDSLWVIAQKFNVTAQQIREKNNLKTDVLQVGQKLVISGKASSSSSSGSSNTTSSTSAKINTMISAAKAQLGVPYRWGGTTPSGFDCSGFIYYVLNKVTSVSRLTAAGYWNTMKSVSQPAVGDFVFFSTYKAGPSHVGIYLGNGEFINANDSGVVISNMNNSYWKQRYLGAKRYF

SEQ ID NO: 6 - protein, 462 aa, Unknown
  LytF protein without signal peptide
ATIKVKSGDSLWKLAQTYNTSVAALTSANHLSTTVLSIGQTLTIPGSKSSTSSSTSSSTTKKSGSSVYTVKSGDSLWLIANEFKMTVQELKKLNGLSSDLIRAGQKLKVSGTVSSSSSSSKKSNSNKSSSSSSKSSSNKSSSSSSSTGTYKVQLGDSLWKIANKVNMSIAELKVLNNLKSDTIYVNQVLKTKSSGSDTSSKDNSSKSNQTSATTKYTVKSGDSLWKIANNYNLTVQQIRNINNLKSDVLYVGQVLKLTGKASSGSSSSSSSSSNASSGTTTTYTVKSGDSLWVIAQKFNVTAQQIREKNNLKTDVLQVGQKLVISGKASSSSSSGSSNTTSSTSAKINTMISAAKAQLGVPYRWGGTTPSGFDCSGFIYYVLNKVTSVSRLTAAGYWNTMKSVSQPAVGDFVFFSTYKAGPSHVGIYLGNGEFINANDSGVVISNMNNSYWKQRYLGAKRYF

SEQ ID NO: 7 - protein, 470 aa, Unknown
  LytF protein with His-Tag without signal peptide
ATIKVKSGDSLWKLAQTYNTSVAALTSANHLSTTVLSIGQTLTIPGSKSSTSSSTSSSTTKKSGSSVYTVKSGDSLWLIANEFKMTVQELKKLNGLSSDLIRAGQKLKVSGTVSSSSSSSKKSNSNKSSSSSSKSSSNKSSSSSSSTGTYKVQLGDSLWKIANKVNMSIAELKVLNNLKSDTIYVNQVLKTKSSGSDTSSKDNSSKSNQTSATTKYTVKSGDSLWKIANNYNLTVQQIRNINNLKSDVLYVGQVLKLTGKASSGSSSSSSSSSNASSGTTTTYTVKSGDSLWVIAQKFNVTAQQIREKNNLKTDVLQVGQKLVISGKASSSSSSGSSNTTSSTSAKINTMISAAKAQLGVPYRWGGTTPSGFDCSGFIYYVLNKVTSVSRLTAAGYWNTMKSVSQPAVGDFVFFSTYKAGPSHVGIYLGNGEFINANDSGVVISNMNNSYWKQRYLGAKRYFLEHHHHHH

SEQ ID NO: 8 - DNA, 26 bp, Unknown
  Attached His-Tag
ctcgagcaccaccaccaccaccactg

SEQ ID NO: 9 - DNA, 1412 bp, Unknown
  LytF protein with His-Tag without signal peptide
gcaacgattaaggtcaaaagcggagattctttatggaaactggcccaaacctataacacaagtgtggcggccctcacatccgccaatcatctttcgactactgttctgtcgatcggccagacgcttactattccaggcagcaaatccagcacttcttcatctacttcaagctcaacaaccaagaagagcggaagttctgtttacacagtgaaaagcggagattcactttggctgatcgcaaatgagtttaaaatgacggtgcaggaactgaaaaaattaaacggactaagcagcgatttaattcgtgctgggcagaaattaaaggtgtccggtactgtttcttcaagctctagttccagtaaaaaaagcaactctaataagagttcaagctccagttcaaaaagcagttctaataagagttcaagttcttcatcttctacgggaacatataaggtgcagcttggagattcactttggaaaattgcaaacaaagtcaatatgtccatcgctgaattgaaggtcttgaacaacttaaaatcagacaccatttacgtgaatcaggtgttgaaaacaaaatcaagcggctctgatacgtcttctaaagacaattcatccaaatcgaaccaaacttcagcaacaactaaatataccgttaaaagcggtgattcactttggaaaatcgcaaacaactataacctgactgtacagcaaatccgaaatatcaacaatctgaaatcagatgtgctttacgttggacaagtattgaagctgacaggtaaagcatcttcaggctcttcatcatcgtcgtcttcttcgtcaaatgcaagctccggcacgacgactacatacacggtgaaaagcggtgattccttatgggtgattgctcaaaaatttaatgtaacagctcagcagattcgtgagaaaaacaatttaaaaacggatgtcttgcaggttggccaaaagctggtcatttccggaaaagcttcatcatcgtcttcatccggttcttcaaacaccaccagctcaacgagtgcgaagattaacacaatgatttcggccgctaaagcgcagcttggggttccgtatcgctggggaggcacgacaccgtccgggtttgactgcagcggattcatttactatgtactgaacaaagtcacatccgtatctagattaacggcagcgggatattggaacacaatgaaatcagttagccagcctgctgtcggagatttcgttttcttttcaacatataaagccggcccttcccacgtcggaatttacctaggcaacggggaattcataaatgccaacgattccggagttgtcatttccaatatgaacaactcttactggaaacagcgctatctcggtgcaaaacgatatttcctcgagcaccaccaccaccaccactg

SEQ ID NO: 10 - DNA, 5307 bp, Artificial Sequence
  pET24d+ plasmid sequence
atccggatatagttcctcctttcagcaaaaaacccctcaagacccgtttagaggccccaaggggttatgctagttattgctcagcggtggcagcagccaactcagcttcctttcgggctttgttagcagccggatctcagtggtggtggtggtggtgctcgagtgcggccgcaagcttgtcgacggagctcgaattcggatccgacccatttgctgtccaccagtcatgctagccatggtatatctccttcttaaagttaaacaaaattatttctagaggggaattgttatccgctcacaattcccctatagtgagtcgtattaatttcgcgggatcgagatctcgatcctctacgccggacgcatcgtggccggcatcaccggcgccacaggtgcggttgctggcgcctatatcgccgacatcaccgatggggaagatcgggctcgccacttcgggctcatgagcgcttgtttcggcgtgggtatggtggcaggccccgtggccgggggactgttgggcgccatctccttgcatgcaccattccttgcggcggcggtgctcaacggcctcaacctactactgggctgcttcctaatgcaggagtcgcataagggagagcgtcgagatcccggacaccatcgaatggcgcaaaacctttcgcggtatggcatgatagcgcccggaagagagtcaattcagggtggtgaatgtgaaaccagtaacgttatacgatgtcgcagagtatgccggtgtctcttatcagaccgtttcccgcgtggtgaaccaggccagccacgtttctgcgaaaacgcgggaaaaagtggaagcggcgatggcggagctgaattacattcccaaccgcgtggcacaacaactggcgggcaaacagtcgttgctgattggcgttgccacctccagtctggccctgcacgcgccgtcgcaaattgtcgcggcgattaaatctcgcgccgatcaactgggtgccagcgtggtggtgtcgatggtagaacgaagcggcgtcgaagcctgtaaagcggcggtgcacaatcttctcgcgcaacgcgtcagtgggctgatcattaactatccgctggatgaccaggatgccattgctgtggaagctgcctgcactaatgttccggcgttatttcttgatgtctctgaccagacacccatcaacagtattattttctcccatgaagacggtacgcgactgggcgtggagcatctggtcgcattgggtcaccagcaaatcgcgctgttagcgggcccattaagttctgtctcggcgcgtctgcgtctggctggctggcataaatatctcactcgcaatcaaattcagccgatagcggaacgggaaggcgactggagtgccatgtccggttttcaacaaaccatgcaaatgctgaatgagggcatcgttcccactgcgatgctggttgccaacgatcagatggcgctgggcgcaatgcgcgccattaccgagtccgggctgcgcgttggtgcggatatctcggtagtgggatacgacgataccgaagacagctcatgttatatcccgccgttaaccaccatcaaacaggattttcgcctgctggggcaaaccagcgtggaccgcttgctgcaactctctcagggccaggcggtgaagggcaatcagctgttgcccgtctcactggtgaaaagaaaaaccaccctggcgcccaatacgcaaaccgcctctccccgcgcgttggccgattcattaatgcagctggcacgacaggtttcccgactggaaagcgggcagtgagcgcaacgcaattaatgtaagttagctcactcattaggcaccgggatctcgaccgatgcccttgagagccttcaacccagtcagctccttccggtgggcgcggggcatgactatcgtcgccgcacttatgactgtcttctttatcatgcaactcgtaggacaggtgccggcagcgctctgggtcattttcggcgaggaccgctttcgctggagcgcgacgatgatcggcctgtcgcttgcggtattcggaatcttgcacgccctcgctcaagccttcgtcactggtcccgccaccaaacgtttcggcgagaagcaggccattatcgccggcatggcggccccacgggtgcgcatgatcgtgctcctgtcgttgaggacccggctaggctggcggggttgccttactggttagcagaatgaatcaccgatacgcgagcgaacgtgaagcgactgctgctgcaaaacgtctgcgacctgagcaacaacatgaatggtcttcggtttccgtgtttcgtaaagtctggaaacgcggaagtcagcgccctgcaccattatgttccggatctgcatcgcaggatgctgctggctaccctgtggaacacctacatctgtattaacgaagcgctggcattgaccctgagtgatttttctctggtcccgccgcatccataccgccagttgtttaccctcacaacgttccagtaaccgggcatgttcatcatcagtaacccgtatcgtgagcatcctctctcgtttcatcggtatcattacccccatgaacagaaatcccccttacacggaggcatcagtgaccaaacaggaaaaaaccgcccttaacatggcccgctttatcagaagccagacattaacgcttctggagaaactcaacgagctggacgcggatgaacaggcagacatctgtgaatcgcttcacgaccacgctgatgagctttaccgcagctgcctcgcgcgtttcggtgatgacggtgaaaacctctgacacatgcagctcccggagacggtcacagcttgtctgtaagcggatgccgggagcagacaagcccgtcagggcgcgtcagcgggtgttggcgggtgtcggggcgcagccatgacccagtcacgtagcgatagcggagtgtatactggcttaactatgcggcatcagagcagattgtactgagagtgcaccatatatgcggtgtgaaataccgcacagatgcgtaaggagaaaataccgcatcaggcgctcttccgcttcctcgctcactgactcgctgcgctcggtcgttcggctgcggcgagcggtatcagctcactcaaaggcggtaatacggttatccacagaatcaggggataacgcaggaaagaacatgtgagcaaaaggccagcaaaaggccaggaaccgtaaaaaggccgcgttgctggcgtttttccataggctccgcccccctgacgagcatcacaaaaatcgacgctcaagtcagaggtggcgaaacccgacaggactataaagataccaggcgtttccccctggaagctccctcgtgcgctctcctgttccgaccctgccgcttaccggatacctgtccgcctttctcccttcgggaagcgtggcgctttctcatagctcacgctgtaggtatctcagttcggtgtaggtcgttcgctccaagctgggctgtgtgcacgaaccccccgttcagcccgaccgctgcgccttatccggtaactatcgtcttgagtccaacccggtaagacacgacttatcgccactggcagcagccactggtaacaggattagcagagcgaggtatgtaggcggtgctacagagttcttgaagtggtggcctaactacggctacactagaaggacagtatttggtatctgcgctctgctgaagccagttaccttcggaaaaagagttggtagctcttgatccggcaaacaaaccaccgctggtagcggtggtttttttgtttgcaagcagcagattacgcgcagaaaaaaaggatctcaagaagatcctttgatcttttctacggggtctgacgctcagtggaacgaaaactcacgttaagggattttggtcatgaacaataaaactgtctgcttacataaacagtaatacaaggggtgttatgagccatattcaacgggaaacgtcttgctctaggccgcgattaaattccaacatggatgctgatttatatgggtataaatgggctcgcgataatgtcgggcaatcaggtgcgacaatctatcgattgtatgggaagcccgatgcgccagagttgtttctgaaacatggcaaaggtagcgttgccaatgatgttacagatgagatggtcagactaaactggctgacggaatttatgcctcttccgaccatcaagcattttatccgtactcctgatgatgcatggttactcaccactgcgatccccgggaaaacagcattccaggtattagaagaatatcctgattcaggtgaaaatattgttgatgcgctggcagtgttcctgcgccggttgcattcgattcctgtttgtaattgtccttttaacagcgatcgcgtatttcgtctcgctcaggcgcaatcacgaatgaataacggtttggttgatgcgagtgattttgatgacgagcgtaatggctggcctgttgaacaagtctggaaagaaatgcataaacttttgccattctcaccggattcagtcgtcactcatggtgatttctcacttgataaccttatttttgacgaggggaaattaataggttgtattgatgttggacgagtcggaatcgcagaccgataccaggatcttgccatcctatggaactgcctcggtgagttttctccttcattacagaaacggctttttcaaaaatatggtattgataatcctgatatgaataaattgcagtttcatttgatgctcgatgagtttttctaagaattaattcatgagcggatacatatttgaatgtatttagaaaaataaacaaataggggttccgcgcacatttccccgaaaagtgccacctgaaattgtaaacgttaatattttgttaaaattcgcgttaaatttttgttaaatcagctcattttttaaccaataggccgaaatcggcaaaatcccttataaatcaaaagaatagaccgagatagggttgagtgttgttccagtttggaacaagagtccactattaaagaacgtggactccaacgtcaaagggcgaaaaaccgtctatcagggcgatggcccactacgtgaaccatcaccctaatcaagttttttggggtcgaggtgccgtaaagcactaaatcggaaccctaaagggagcccccgatttagagcttgacggggaaagccggcgaacgtggcgagaaaggaagggaagaaagcgaaaggagcgggcgctagggcgctggcaagtgtagcggtcacgctgcgcgtaaccaccacacccgccgcgcttaatgcgccgctacagggcgcgtcccattcgcca

SEQ ID NO: 11 - protein, 8 aa, Unknown
  NlpC/P60 domain sequencepart 1
GVPYRWGG

SEQ ID NO: 12 - protein, 8 aa, Unknown
  NlpC/P60 domain sequencepart 2
GVPYRWGA

SEQ ID NO: 13 - protein, 8 aa, Unknown
  NlpC/P60 domain sequencepart 3
GVPYKWGG

SEQ ID NO: 14 - protein, 8 aa, Unknown
  NlpC/P60 domain sequencepart 4
GVPYKWGA

SEQ ID NO: 15 - protein, 7 aa, Unknown
  NlpC/P60 domain sequencepart 5
GFDCSGF

SEQ ID NO: 16 - protein, 7 aa, Unknown
  NlpC/P60 domain sequencepart 6
GIDCSGF

SEQ ID NO: 17 - protein, 7 aa, Unknown
  NlpC/P60 domain sequencepart 7
GFDCSAF

SEQ ID NO: 18 - protein, 7 aa, Unknown
  NlpC/P60 domain sequencepart 8
GIDCSAF

SEQ ID NO: 19 - protein, 7 aa, Unknown
  NlpC/P60 domain sequencepart 9
AFDCSGF

SEQ ID NO: 20 - protein, 7 aa, Unknown
  NlpC/P60 domain sequencepart 10
AIDCSGF

SEQ ID NO: 21 - protein, 7 aa, Unknown
  NlpC/P60 domain sequencepart 11
AFDCSAF

SEQ ID NO: 22 - protein, 7 aa, Unknown
  NlpC/P60 domain sequencepart 12
AIDCSAF

SEQ ID NO: 23 - protein, 9 aa, Unknown
  NlpC/P60 domain sequencepart 13
PAVGDFVFF

SEQ ID NO: 24 - protein, 7 aa, Unknown
  NlpC/P60 domain sequencepart 14
VGDFVFF

SEQ ID NO: 25 - protein, 7 aa, Unknown
  NlpC/P60 domain sequencepart 15
VGDLVFF

SEQ ID NO: 26 - protein, 7 aa, Unknown
  NlpC/P60 domain sequencepart 16
HVGIYLG

SEQ ID NO: 27 - protein, 7 aa, Unknown
  NlpC/P60 domain sequencepart 17
HMGIYLG

SEQ ID NO: 28 - protein, 7 aa, Unknown
  NlpC/P60 domain sequencepart 18
HVGIYIG

SEQ ID NO: 29 - protein, 7 aa, Unknown
  NlpC/P60 domain sequencepart 19
HVGIYLN

SEQ ID NO: 30 - protein, 7 aa, Unknown
  NlpC/P60 domain sequencepart 20
HMGIYIG

SEQ ID NO: 31 - protein, 7 aa, Unknown
  NlpC/P60 domain sequencepart 21
HMGIYLN

SEQ ID NO: 32 - protein, 7 aa, Unknown
  NlpC/P60 domain sequencepart 22
HVGIYIN

SEQ ID NO: 33 - protein, 4 aa, Unknown
  NlpC/P60 domain sequencepart 23
FINA

SEQ ID NO: 34 - protein, 4 aa, Unknown
  NlpC/P60 domain sequencepart 24
FVNA

SEQ ID NO: 35 - protein, 4 aa, Unknown
  NlpC/P60 domain sequencepart 25
FANA

SEQ ID NO: 36 - protein, 4 aa, Unknown
  NlpC/P60 domain sequencepart 26
FIHA

SEQ ID NO: 37 - protein, 4 aa, Unknown
  NlpC/P60 domain sequencepart 27
FVHA

SEQ ID NO: 38 - protein, 4 aa, Unknown
  NlpC/P60 domain sequencepart 28
FAHA

SEQ ID NO: 39 - protein, 7 aa, Unknown
  NlpC/P60 domain sequencepart 29
GLDCSGF

SEQ ID NO: 40 - protein, 7 aa, Unknown
  NlpC/P60 domain sequencepart 30
GLDCSAF

SEQ ID NO: 41 - protein, 7 aa, Unknown
  NlpC/P60 domain sequencepart 31
ALDCSGF

SEQ ID NO: 42 - protein, 7 aa, Unknown
  NlpC/P60 domain sequencepart 32
ALDCSAF